European Patent Specification EP 4 013 434 B1, published October 23, 2024. Title: Bacterium comprising myo-inositol to propionate pathway. Applicant: Wageningen Universiteit. The sequence listing filed with the application follows.

SEQUENCE LISTING (48 sequences)

SEQ ID NO: 1 - DNA, 1014 bp, Anaerostipes rhamnosivorans
atggtaaatgtaggtattatcggagcaggaagaatcggaagagtacatgtagaaagcatctgcacacaggtaggaaacgcaaaggttaagactcttgctgatccttttatgtcagaggacacagcagtatgggcaaaagaaatgggtgttgaaaataccaccaaagattacaaagacatcttaaatgatcctcagatcgacgcagtgctgatctgctcatccacagatacacattcaccgatctccgtagaggctattgaagcaggaaaacatgtattctgcgaaaagccaatcgaccatgacgtacagaagattcaggaagtagtcgacgctttaaagaaaagcgacgtaaaataccaggtaggattcaaccgccgttttgaccataactttgaagccatccgggatgccgtggctgctggaaagattggtgagacacagatcatcaaagttacatccagagatcctgaaccgccaagtgctgattatgtaaaagtttccggaggaatgttcctggacatgacaatccatgattttgacatggtccgtttccttgcaggatgtgacgctgaagaagtgtatgtagaagctgcagtccttgtagatcctgccatcggtgaagccggagatgtggacactgctgttatcacattaaaaatgaaaaacggttccatcgccgtgattgacaactcaagaaaagccgtttacggatacgatcagagagctgaagtgttcggatcaaagggaatggtcgtaacagcaaacgattccgcatcctcagccgtgatcagtaatgcggacggagtgacaggagaaaaacctctttacttcttcctggaacgctacatggcagcctatgcaaaagaaatcaaatgctttatcgacgccatcgaaaaaaacacagacacccctcttggagttatggacggtcttgagccagtacttatggggcttgcggctaaaaaatcattagaagaacaccgcccagtaaaaatttctgaaattacagtatag

SEQ ID NO: 2 - protein, 337 aa, Anaerostipes rhamnosivorans
MVNVGIIGAGRIGRVHVESICTQVGNAKVKTLADPFMSEDTAVWAKEMGVENTTKDYKDILNDPQIDAVLICSSTDTHSPISVEAIEAGKHVFCEKPIDHDVQKIQEVVDALKKSDVKYQVGFNRRFDHNFEAIRDAVAAGKIGETQIIKVTSRDPEPPSADYVKVSGGMFLDMTIHDFDMVRFLAGCDAEEVYVEAAVLVDPAIGEAGDVDTAVITLKMKNGSIAVIDNSRKAVYGYDQRAEVFGSKGMVVTANDSASSAVISNADGVTGEKPLYFFLERYMAAYAKEIKCFIDAIEKNTDTPLGVMDGLEPVLMGLAAKKSLEEHRPVKISEITV

SEQ ID NO: 3 - DNA, 1020 bp, Anaerostipes rhamnosivorans
atgaacaaagtaagagtaggtattgctggtttaggaagattagggaaattacatgcagagaatatcgcattcaagattccaaacgcggaacttacagcggcctgttcgatcgcgccagaggaattggaatatgccacagaacatttcggggtaaccgatgtttatacagatttttatgagatgttagataaagcagacattgatgtcgtggcggtggtgaccacgagcggagaacactgctggcagatcaaagcagcattggacgctggaaaacatgttttttgcgataaacctctcggggttacggtcaatgaatgtaaaacagcggaggccgcggtggaacgccacccagagcttacattttttcttggatttatgcgccgttatgacccatcctacgcttatgcgaaaaagaaaatccaggagggagccattggtaagccgtatatggtaaaagcggcagggatcgacccggaagctctggtggagggagcagtaaaatttgcagccaccagcggcggtatttttatcgacatggcaatccatgatatcgatttaatgcgctggcttttggaatccgatccggtggaagtctacgctgcaggggccacgtttaaacatcccgaattcagggaggcaggggatgacgagacgggggcagccatgtacaaatgtgagaacggtgcactgggatttgtacatgttgggcgtacagcggcccatggatatcatgtggagacagagatcatcggaacagagggaagcctgagaatcagtcctgtaccggaaaagaacctgtgtatgatctacgatgagaacggagctgtgacagaatgtgtcagcggttttgcagaacggtttgcagaggcatacctgttggaaatgaaggaattcatcaactgtgtccagagcggcacaaagccggatgtgaccgtatatgacggcacaaaatccacacagatcggttttgccacaacagaagcgtggaaaaagggctgtactgcaaagatccagtactag

SEQ ID NO: 4 - protein, 339 aa, Anaerostipes rhamnosivorans
MNKVRVGIAGLGRLGKLHAENIAFKIPNAELTAACSIAPEELEYATEHFGVTDVYTDFYEMLDKADIDVVAVVTTSGEHCWQIKAALDAGKHVFCDKPLGVTVNECKTAEAAVERHPELTFFLGFMRRYDPSYAYAKKKIQEGAIGKPYMVKAAGIDPEALVEGAVKFAATSGGIFIDMAIHDIDLMRWLLESDPVEVYAAGATFKHPEFREAGDDETGAAMYKCENGALGFVHVGRTAAHGYHVETEIIGTEGSLRISPVPEKNLCMIYDENGAVTECVSGFAERFAEAYLLEMKEFINCVQSGTKPDVTVYDGTKSTQIGFATTEAWKKGCTAKIQY

SEQ ID NO: 5 - DNA, 900 bp, Anaerostipes rhamnosivorans
atgtttaacaaagaaaaagtaaaattaggaattgccccgatcgcttggaccaacgatgatcttccggatcttggaaaagaaaacacctttgagcagtgtgtcagtgaaatggcattggcagggtacactggttccgaagtaggaaataaatatccaaaggacccagaggttctaaaaaaggccctgaaactccggggaatggagatctgcaatcagtggttctcatcatttttgatcacaaagccatttgaagaggtggaaaaagagttccgcgctcaactgagtttcttaaaggctgtgggagcaaagatcattggtgcttctgaacagagccacagtgtacagggtatgctggatactccgatctttggacataagtatgtgatgaatgacgaagagtgggaaaccttctgtacgggaatgaataagttaggaaaaatcgcaaaagaagaatacggcatcagcttaaccttccaccatcatatgggaactgtggtacaggacccggatgaagtggaaagaatgatggcaaacacagatcctgaatatgtgaatctgttatttgatacagggcattttacatactgcggggcagatcctcttgaaatggtgaaaaaatatgtggaccgcatcaaacatgtccatcttaaggatatccgtccggaaatcgtagaaaaagtgaaagcagaaaacttaagcttcttagatggtgtgcgtatgggggcgtttacggtaccgggtgacggatgtattgattttgatccgatctttaaggtgcttgaagattcaggatatgaaggatatatgctggtagaggcagaacaggatccggccaaggcaaatccgcttgaatatgccatgaaggcaagaaaattcatcgctgagaaaactggattataa

SEQ ID NO: 6 - protein, 299 aa, Anaerostipes rhamnosivorans
MFNKEKVKLGIAPIAWTNDDLPDLGKENTFEQCVSEMALAGYTGSEVGNKYPKDPEVLKKALKLRGMEICNQWFSSFLITKPFEEVEKEFRAQLSFLKAVGAKIIGASEQSHSVQGMLDTPIFGHKYVMNDEEWETFCTGMNKLGKIAKEEYGISLTFHHHMGTVVQDPDEVERMMANTDPEYVNLLFDTGHFTYCGADPLEMVKKYVDRIKHVHLKDIRPEIVEKVKAENLSFLDGVRMGAFTVPGDGCIDFDPIFKVLEDSGYEGYMLVEAEQDPAKANPLEYAMKARKFIAEKTGL

SEQ ID NO: 7 - DNA, 1932 bp, Anaerostipes rhamnosivorans
atgagtacaaccagaatgacagtagcacaggctcttgtaaaattccttgacaatcagtatgtggaatttgacggggaagaaacaaaatttgtagaaggtttctttactatcttcggacacgggatcgccgttggtctcggagaggcattggacagcaatcctgggagcttaaaggttcttcagggaagaaatgagcagggaatgtgccacgtagcgacagcttacgcaaaacaaaatagaagaaggaagatcattccttgtgcatcttctgtaggacccggagcggcaaatatggtgacagcagcggctacagctacagtgaacaatattccgcttttggtagtgccttctgacacatttgccacaagacagccggacccggtgctccagcagttagaaaagagtgacagtctctctacaacaacaaacgacgcattcaaaccggtttgtaaatattgggataggatcatccgcccggaacagctgatgacagccatggtcaacgctatgcgtgttctcacagatccgtcagagacaggcgctgtgtgcattgcactctcccaggatgtagaaggagaatcttatgatttccctgactatctgtttgaaaaacgtgtacataggatcacaagaccttgcgcggtaaaagaagagatcgaggaccttgtaaaagtcattaaagaagcgaaaaatccgttagtgatcgtgggcggaggtgtgaagtattctgaggcaggagaagctgtagaaaagttctgcgaagactttaacatcccgttcggagagagccaggcaggaaaaagtgcctgcaagtcaagccacccttactgcttaggaggaatcggcgtcacaggaaccctggctgccaataccatcgctgatgaagctgatgtggtcattgcagtgggaaccagactttcagactttacaacaggatctaaaggacagttcaaaaatcctaatgtaaaaatggtgacgatcaacaacaataaatatcatgcatataaaatggatgcagtaaaagctgtcggagacgcgaaagtgacagtggaagctctttctgctagactgaaagaggaaggatacaagtctgcttacacaacagagatccaggacgcaaaggcagcctgggataaagaaatggaccgccttgcgaatattgagtatacaggcgatgactttgagccggagatcaaagcgagagatccgcgtacgattcctgaattcgtaaaacttacagggggacttatcactcagactgcagcattgtgcaaaatccgtgaggtcattgatgaagacgctaatattgtgacagcaggggggagtcttccaagctgtatgcagagaatctggaccacagacaaacgaggcggatatcacgcagaatacggatattcctgcatgggatatgaagtggcgggagcgctcggcgtaaagatggcagagcctgagcatgaatcctacgtggttgtgggggatgccagctttcagatgctccacagtgagattatgacagcgatgcaggaaaaacaaaagatcaacatccttgtatttgacaactgcggatttggctgtatcaacaaccttcagatgaatcatggagtgggaagtcttgcaacagagttcagataccgcgatgaaaacaatgagatcaagggtgatctgatcccggttgactatgcaaaagtcggagaaggatacggactcaagacgtacagtgtaagaacgatcaaagagctggaggaagcattgatcgatgctaagaaacaggacgttgccacattgatcgacttgaaggtcattccgaaaacaatgacagacggttacaaatcatggtggaacgtaggtattgcgacaacttctgtgaaagaaagcgtgcagaaagcatgtgaaggagtattggaaggccgcaaaaacgcaagacagtattag

SEQ ID NO: 8 - protein, 643 aa, Anaerostipes rhamnosivorans
MSTTRMTVAQALVKFLDNQYVEFDGEETKFVEGFFTIFGHGIAVGLGEALDSNPGSLKVLQGRNEQGMCHVATAYAKQNRRRKIIPCASSVGPGAANMVTAAATATVNNIPLLVVPSDTFATRQPDPVLQQLEKSDSLSTTTNDAFKPVCKYWDRIIRPEQLMTAMVNAMRVLTDPSETGAVCIALSQDVEGESYDFPDYLFEKRVHRITRPCAVKEEIEDLVKVIKEAKNPLVIVGGGVKYSEAGEAVEKFCEDFNIPFGESQAGKSACKSSHPYCLGGIGVTGTLAANTIADEADVVIAVGTRLSDFTTGSKGQFKNPNVKMVTINNNKYHAYKMDAVKAVGDAKVTVEALSARLKEEGYKSAYTTEIQDAKAAWDKEMDRLANIEYTGDDFEPEIKARDPRTIPEFVKLTGGLITQTAALCKIREVIDEDANIVTAGGSLPSCMQRIWTTDKRGGYHAEYGYSCMGYEVAGALGVKMAEPEHESYVVVGDASFQMLHSEIMTAMQEKQKINILVFDNCGFGCINNLQMNHGVGSLATEFRYRDENNEIKGDLIPVDYAKVGEGYGLKTYSVRTIKELEEALIDAKKQDVATLIDLKVIPKTMTDGYKSWWNVGIATTSVKESVQKACEGVLEGRKNARQY

SEQ ID NO: 9 - DNA, 786 bp, Anaerostipes rhamnosivorans
atgggtaaagtattcggctatcctgagtttgatgtaaacggggaaaaggttttaacaacatatgacaatgattataaagaaatgctgatggacatccgcgtcttccgcttaaaagcgggagatgtgaagaccttctgcaaagaaaaagaggagaccgcggttcttttactaaaaggggatgtcgtattctcatttgatgaaacttccaaagaagtcacaagaaaagatgtatttacagaaggaccttgggcagtacatatctgcacaggagccaaagtcatagtggaagcaaaggcagactctgaaatcttggtacagtccacaatgaatgaccagacatttgagagtaaattgtatgcgccggaagatgctccttggggatattcctgtgtaggaaagttcggaaatgtggctaaacgccgtgtcaataccatctttgaccatgacattgcaccatactccaacatggtattaggtgaagtcttaaatgaccgcggaaactggtcaggatatcttcctcacagacatccgcagccggaaacttattacttcctgtttgaccatccggaaggatttggggcaagctttgtgggagaccaggtatttaagagtacagacggaagcttctcagcgattccagggggagaacttcatcctcaggcagtggctccgggataccaaatgtatacttgctggatgatccgtcatctggaagggaacccatggcttcagacagacagaaatgaagacgaacgctacgtttggcttcatgacgcagaattctaa

SEQ ID NO: 10 - protein, 261 aa, Anaerostipes rhamnosivorans
MGKVFGYPEFDVNGEKVLTTYDNDYKEMLMDIRVFRLKAGDVKTFCKEKEETAVLLLKGDVVFSFDETSKEVTRKDVFTEGPWAVHICTGAKVIVEAKADSEILVQSTMNDQTFESKLYAPEDAPWGYSCVGKFGNVAKRRVNTIFDHDIAPYSNMVLGEVLNDRGNWSGYLPHRHPQPETYYFLFDHPEGFGASFVGDQVFKSTDGSFSAIPGGELHPQAVAPGYQMYTCWMIRHLEGNPWLQTDRNEDERYVWLHDAEF

SEQ ID NO: 11 - DNA, 1017 bp, Anaerostipes rhamnosivorans
atgaagtatgttgaatttgaccagacaagaccaatggatttagtactcatcggaagggtagccatcgattttaacccggtagattatttccacccgttatctgagtgcactaccttcaagaagtatgtgggaggatctccggcaaacatcgcagtgggcatcacaaggcacggaaagaaagccggattcatcggcaaagtttctgatgaccagttcggagagtatgtagtagacttcttcaataaagagggaatcgatacatcccatattacaaaatgtacgaacggagaaaagcttggacttacctttacagaaattctttccagagaagaaagcagcatcttaatgtaccgcaactgcatcgcagacttacagttatctgtggatgacattgacgaagaatacataaagaacacaaaagcaatcctggtttccggaacagcattggcacagagcccatccagggaagcagtgttaaaagcagtgatgcttgccaagaaaaatgatacaaagatcatctttgacattgactatagagaatacaactggaaaaattccgatgagatttcaatctactattctttagtagccagagaagcagatatcatcatgggatctagagaagaatttgacctgacagaaaaactgataaaaccgggcagaacagacaaagaatctgcacaggcatggaacactgaaaatgcaaagatcgttgtcatcaaacatggcaaaaaaggatctacagcatataccaatgacggaaatgactattcaatcaaaccgttcccggttgaggcgttaaaaggctttgggggcggagacggatatgcatccggcttcttatatggaatatttgaaggatgggatatgatcgagtgtctggaattcggaagtgcggaagcggccatgatggtgagaagccattcttgttctgaagaacttccaaaccctcaggaagtcaaagactttatccgcgagacaaaagacaaatatggcgaaatgattgcgagagtatag

SEQ ID NO: 12 - protein, 338 aa, Anaerostipes rhamnosivorans
MKYVEFDQTRPMDLVLIGRVAIDFNPVDYFHPLSECTTFKKYVGGSPANIAVGITRHGKKAGFIGKVSDDQFGEYVVDFFNKEGIDTSHITKCTNGEKLGLTFTEILSREESSILMYRNCIADLQLSVDDIDEEYIKNTKAILVSGTALAQSPSREAVLKAVMLAKKNDTKIIFDIDYREYNWKNSDEISIYYSLVAREADIIMGSREEFDLTEKLIKPGRTDKESAQAWNTENAKIVVIKHGKKGSTAYTNDGNDYSIKPFPVEALKGFGGGDGYASGFLYGIFEGWDMIECLEFGSAEAAMMVRSHSCSEELPNPQEVKDFIRETKDKYGEMIARV

SEQ ID NO: 13 - DNA, 837 bp, Anaerostipes rhamnosivorans
atggcattagtcaaaatgaaacagttattagagcaggcaaaaaaggaaaacagaggatgcggtgcattcagtgtgggcaatatggaaatggtcaaaggggcgattcaggcagcggaggagatgaatacaccgatcatcctgcagatcgctgaagtgcggctcgcccattcaccgcttcatcttatggggccgatgatggtgcaggcggcaaaagaggcaaaggtggatgtggcagttcatctggaccacggacttaacattgagactgtaaaaaaagcgctggaactgggatttacctctgttatgctggatgcatccagagattcgtttgaagaaaatatcagaaaaacaaaagaagttgtcgctctggcagcacagtacggagcaaccgtggaagcggaattagggctggtaggcggaagcgaagacggaaagagtgaccatggaatccagtgcaccaagcctcaggacgccaaggtcttctgtgagcagaccggagtggatgccctggccgttgccattggaaatgcccacggggactatccggtagctccgactttggaatttggtgtattggaagacattcacaatattactgccaaaccattggtgcttcacggcggaagcggtattacagatgaggatttcagaaaagccatctctcttggaatctgcaaagtgaacattgcaactgcaagctttaacagcctgacaaaagaagtggaaaactatctggagacagaaggaaaacataattacttcgatatgaacgaagctatggtaaagggtgtctatgacaacgtaaaacgccatatccagatctttaactgcagataa

SEQ ID NO: 14 - protein, 278 aa, Anaerostipes rhamnosivorans
MALVKMKQLLEQAKKENRGCGAFSVGNMEMVKGAIQAAEEMNTPIILQIAEVRLAHSPLHLMGPMMVQAAKEAKVDVAVHLDHGLNIETVKKALELGFTSVMLDASRDSFEENIRKTKEVVALAAQYGATVEAELGLVGGSEDGKSDHGIQCTKPQDAKVFCEQTGVDALAVAIGNAHGDYPVAPTLEFGVLEDIHNITAKPLVLHGGSGITDEDFRKAISLGICKVNIATASFNSLTKEVENYLETEGKHNYFDMNEAMVKGVYDNVKRHIQIFNCR

SEQ ID NO: 15 - DNA, 747 bp, Anaerostipes rhamnosivorans
atgcgtaaaacaatcgtagcaggaaactggaaaatgaacaaaacacctagcgagacagtagctttagttaatgaattaaagccattggtagcaagcgaggtttcagatgttgtcttctgtgtgccggccatctgtattccggcagcactggaagctgcaaaaggaagtaacatcaacatcggcgctgagaacatgtattttgaagagagcggcgcttacacaggcgagatcgctccgaatatgttaacagacttaggtgtgaaatatgttatcatcggacattctgagagaagagaatattttgcagaaacagatgagacagtgaataaaaaagtcttaaaagcttttgaacatggaattactccaatcgtttgctgcggtgagacacttgctcagagagagcagggtgtgaccatcgatttcgtacgccagcagatcaagatcgcattccagggtgtgactgctgaccaggcaaagacagctgtcattgcatacgaaccgatctgggctatcggaacaggaaaagttgcgacgacagaacaggctcaggaagtatgtaaagcgatccgtgagtgcatcgctgaagtatacgatcaggcaacagcggacgctattcgtatccagtacggcggttctgtatccgctgcaagtgcaccagaattatttgcacaggaagacatcgatggaggattagtcggtggagctgctttaaaaccagactttggtaagatcgtgaattacaaataa

SEQ ID NO: 16 - protein, 248 aa, Anaerostipes rhamnosivorans
MRKTIVAGNWKMNKTPSETVALVNELKPLVASEVSDVVFCVPAICIPAALEAAKGSNINIGAENMYFEESGAYTGEIAPNMLTDLGVKYVIIGHSERREYFAETDETVNKKVLKAFEHGITPIVCCGETLAQREQGVTIDFVRQQIKIAFQGVTADQAKTAVIAYEPIWAIGTGKVATTEQAQEVCKAIRECIAEVYDQATADAIRIQYGGSVSAASAPELFAQEDIDGGLVGGAALKPDFGKIVNYK

SEQ ID NO: 17 - DNA, 1017 bp, Anaerostipes rhamnosivorans
atggcagtaaaagtagcgattaatggatttggacgtattggacgtcttgcattcagacagatgttcggagcagaaggttatgaagttgtagcaatcaacgatttaacaaatcctaagatgttagcacatttattaaagtatgattctgcacagggaagatatgcattaggcgacaaggtagaagcaaaagaatcttccatcgtagttgacggaaaagaaatcgaaatctacgcagaagcagacgcaacaaaacttccttggggagaattagatgttgatgttgtattagaatgtacaggattctacacatctaaagacaaagcatccgcacacgttcaggcaggagctaagaaagttgttatttctgcgccagctggaaatgatcttccaactatcgtatataatgtaaaccacgatacattgacaaaagaagacacagtcatctcagcagcatcttgtacaacaaactgcttagcacctatggctgatgcactgaacaagtatgcaccaatccagtctggtatcatgttaacagtacatgcttacacaggagatcagatgactcttgacggacctcagagaaaaggtgacttaagaagagcacgtgcagctgcagtcaacatcgtacctaactctacaggtgctgcaaaagctatcggattagttatcccagaattaaacggaaaattaatcggatctgctcagcgtgtaccggttcctacaggatcaacaacacttttaacagcagttgttaaaggtgacaatgtaactgttgaaggaatcaacgcagctatgaaagcagcagcaacagagtctttcggatacacagaagaagaattagtatcttctgacatcatcggaatcaaatatggttctttattcgacgcaactcagacaatggttactgaagttggtgacggattatatgaagtacaggttgtttcttggtatgacaacgaaaactcatacacaagccagatggttagaacaatcaaatactttgcagaattagcataa

SEQ ID NO: 18 - protein, 338 aa, Anaerostipes rhamnosivorans
MAVKVAINGFGRIGRLAFRQMFGAEGYEVVAINDLTNPKMLAHLLKYDSAQGRYALGDKVEAKESSIVVDGKEIEIYAEADATKLPWGELDVDVVLECTGFYTSKDKASAHVQAGAKKVVISAPAGNDLPTIVYNVNHDTLTKEDTVISAASCTTNCLAPMADALNKYAPIQSGIMLTVHAYTGDQMTLDGPQRKGDLRRARAAAVNIVPNSTGAAKAIGLVIPELNGKLIGSAQRVPVPTGSTTLLTAVVKGDNVTVEGINAAMKAAATESFGYTEEELVSSDIIGIKYGSLFDATQTMVTEVGDGLYEVQVVSWYDNENSYTSQMVRTIKYFAELA

SEQ ID NO: 19 - DNA, 1194 bp, Anaerostipes rhamnosivorans
atgttaaacaagaaatcagtagatgatatcaacgtaaaaggaaaaaaagtcttagtgcgctgtgacttcaacgttccgcttcaggatggaaagatcacagatgagaaccgtcttgtggcagcacttcctacactaaagaagttaattgctgacggcggaaagctgatcctctgctcacacttaggaaaaccaaaaggggaaccgaaaccggagttatctcttgcgccagtagcagaaagattaagcgagttattaggacaggaagtaaagtttgctgcagatgacaacgtggtaggaccgaatgcaaaagctgcggtagaaggaatgcaggacggggatgtcattttacttcagaatacacgctacagagcagaagagacaaagaatggagaagagttcagcaaagaacttgcaagtctctgcgatgtttttgttaatgatgcttttggtaccgctcatagagctcactgctctaacgtgggagttacaaagttcgtggacactgcagttgtaggatatttaatgcagaaagagattgatttcttaggaaatgcggtcaacaatccggaacgtcctatggtcgctatcttgggaggagcaaaggtttcctctaagatctctgtgatcaataacctgctagacaaagtcgatactttgatcatcggcggaggtatggcatatactttcatgaaagcattgggagaagaagttggagattcccttctggaagctgactacttagactacgcaaaagaaatgatggacaaggcaaaagaaaaaggtgtgaacttactgattcctgttgacactgtagttgctgatgacttctcaaatgacgccaacatcaaaactgttgagagaggcggaatcgaagcaggatggcagggacttgacatcggaccaaagacaagagaactgttttcaaatgcactgaaagatgccaagactgtagtatggaacggaccgatgggatgctttgagatgccgaactttgcagcaggaaccgttgcagttgcagaagcactggcagagatcgacgctacaactatcattggcggaggagattccgcagcggcagttaaccagctcggattcggagataagatgactcatatctctacaggtggtggagcatcactggaattcctggaaggaaaagaattaccaggcgttgcagcggcaaacgataaataa

SEQ ID NO: 20 - protein, 397 aa, Anaerostipes rhamnosivorans
MLNKKSVDDINVKGKKVLVRCDFNVPLQDGKITDENRLVAALPTLKKLIADGGKLILCSHLGKPKGEPKPELSLAPVAERLSELLGQEVKFAADDNVVGPNAKAAVEGMQDGDVILLQNTRYRAEETKNGEEFSKELASLCDVFVNDAFGTAHRAHCSNVGVTKFVDTAVVGYLMQKEIDFLGNAVNNPERPMVAILGGAKVSSKISVINNLLDKVDTLIIGGGMAYTFMKALGEEVGDSLLEADYLDYAKEMMDKAKEKGVNLLIPVDTVVADDFSNDANIKTVERGGIEAGWQGLDIGPKTRELFSNALKDAKTVVWNGPMGCFEMPNFAAGTVAVAEALAEIDATTIIGGGDSAAAVNQLGFGDKMTHISTGGGASLEFLEGKELPGVAAANDK

SEQ ID NO: 21 - DNA, 606 bp, Anaerostipes rhamnosivorans
ttgaagttatatatgatgaggcacggagaaactccatggaataaagtgcggaggattcaggggcagtcagacgtggatctgagtgaagcgggcagggaagcagccaggctcaccaggagagcactgaaagatttccattttgatgcggcctacacgagcccgctgagcagagcgagagaaacaggggagatcatcctggagggcagagggatccctctgctggaggatgaacggcttaaggaggccaacttcggaccttatgaaggggcacacatcaatgaattatatgaaagagaagaaccgattctggatttctttgaccggccggaacagatggcctatattgaaggagcggagactccggctcaggtagtagaaagatccaggatatttttagaggaatttatacttccgatggaaaaagaagcagaaagtgtgatcttatttacccacggagctttcatccacgggatgctgactaatatgtatcaaagagagatcagggacttttggaaaggaccgaagcttaagaattgttctatcagtacggctgaagtcagggacggtcagttccgcattttgagtgaggctgaggtcttttactga

SEQ ID NO: 22 - protein, 201 aa, Anaerostipes rhamnosivorans
MKLYMMRHGETPWNKVRRIQGQSDVDLSEAGREAARLTRRALKDFHFDAAYTSPLSRARETGEIILEGRGIPLLEDERLKEANFGPYEGAHINELYEREEPILDFFDRPEQMAYIEGAETPAQVVERSRIFLEEFILPMEKEAESVILFTHGAFIHGMLTNMYQREIRDFWKGPKLKNCSISTAEVRDGQFRILSEAEVFY

SEQ ID NO: 23 - DNA, 1284 bp, Anaerostipes rhamnosivorans
atggattatttagagattgaaaaggtcataggaagggaaattattgattccaggggaaatcctacagtggaagcagaagttcttttagccggcgggacaatcggacggggcacagcacccagcggagcttcaactggagaatttgaggcgttggaattaagagacggagataaggagcgttttggaggaaaaggtgtgtccaaggcagttcataatattaatacgatcattaacgatactttaaaagggatggatgcatccgatacttacgcggtggacagagcgatgatcagcgtagacggaacaaaggataaatcaaagcttggggccaatgcgatccttgcggtttcgattgcatgcgcaaaggcggcatcggcaggcctggatctgccattataccgttttctgggcggtgttaatgccaaccgtcttccggtgccgatgatgaacattttaaacggaggtgcccatgcggccaacaccgtcgatgtacaggagtttatgatcatgcctgtgggagcagaaaatttcagggaagcactccggtggtgtacggaagtattccacgccttggcagctttgctgaaatccaaagggctggcaacctccgtgggtgatgaaggcgggtttgcgcctgaccttgcaagtgatgaggaagccatcgaatatattttggaagctgttcaggcagcgggatatgagccgggcagtgattttgttctggctatggatgctgcttccagcgagtggaaaggcgcgaacaaaggtgaatatattcttcctaagagtggcaagaaatttacctcagaagaactggtggaccactggaaatcactttgtgagaaatatccgatcagctccattgaggatggattggatgaggaagactgggacggctggaaatacatgacccaggagcttggagagaaaatccagctggtgggagatgacttatttgtaacgaatacggaacgccttggaaaaggtatcaagatgggatgcggaaattctatcttgatcaagctgaaccagatcggttctgtgtcggagacattggaagctattaagatggcccataaagcgggttacacagcggtcacatcccaccgttcaggggagacagaagacacgaccatcgcagatctcgctgttgcacttaataccggacagatcaaaaccggtgcaccgagcagaagtgagagggtggcaaaatataatcagcttctgaggattgaagaggaactgggggaaagtgccgtatacccgggagtcggaacattttag

SEQ ID NO: 24 - protein, 427 aa, Anaerostipes rhamnosivorans
MDYLEIEKVIGREIIDSRGNPTVEAEVLLAGGTIGRGTAPSGASTGEFEALELRDGDKERFGGKGVSKAVHNINTIINDTLKGMDASDTYAVDRAMISVDGTKDKSKLGANAILAVSIACAKAASAGLDLPLYRFLGGVNANRLPVPMMNILNGGAHAANTVDVQEFMIMPVGAENFREALRWCTEVFHALAALLKSKGLATSVGDEGGFAPDLASDEEAIEYILEAVQAAGYEPGSDFVLAMDAASSEWKGANKGEYILPKSGKKFTSEELVDHWKSLCEKYPISSIEDGLDEEDWDGWKYMTQELGEKIQLVGDDLFVTNTERLGKGIKMGCGNSILIKLNQIGSVSETLEAIKMAHKAGYTAVTSHRSGETEDTTIADLAVALNTGQIKTGAPSRSERVAKYNQLLRIEEELGESAVYPGVGTF

SEQ ID NO: 25 - DNA, 3525 bp, Anaerostipes rhamnosivorans
atggcaagaaaaatgaaaaccatggatggtaacacagctgcagcacacgtgtcttacgcttttactgagacagctgctatctacccaattacaccatcctcaccaatggcagaatcaacagaccagtgggcaacacagggaaagaaaaatattttcggacatcctgtaaaattagttgaaatgcagtcagagggcggagcagcaggaactgttcacggatctcttgcagcaggcgcattgacaactacatacactgcatctcagggattattactgatgattcctaatatgtacaagatcgcaggtgaattaatgccttgtgtatttgatgtatctgcacgtgcaatcgcatctcatgcactgaatatctttggtgatcactctgacgtttacgcttgtcgccagacaggttttgcaatgctttgcagctccagcgttcaggaagttatggacttaggcgctgttgctcatttatctacaatcaagggaagcgttccagttctccatttcttcgatggattcagaacatctcatgagatccagaagattgaaatgtgggacaacgaagatcttgcagatatggtagattacgatgctcttgaaaagttcagagcaaatgctttgaatccagaacatccggttctccgcggatctgctcagaatccagatatcttcttccaggcaagagaagcatgcaacaaatactacgatgcattcccggcaatcgtcgaagattacatgaaccaggttaatgcaaagatcggtacagattataaattattcaactactacggagctgctgatgctgaatctgttatcattgcaatgggatctgtatgtgagactatcgatgagaccatcgattacttaacagcaaaaggcgaaaaagtcggtgttgttaaagtaagactttacagaccattcgtagctgaaaaattactcgaagttatcccagagactgttaaaacaatcaacgttttagacagaacaaaagaaccgggatctcttggagagccattatacttagacgttgtttctgcattaagaggaacaaaattcgagcaggtaacaatcaacggaggacgttacggattaggatccaaagatacaactcctgctgatatcatctctgtattcaataacaaagataagaaagaattcacagttgcgatcaacgatgatgtgacaaacttatctcttgaaagaggagaagctgtttcttctacaccagaaagcacagtaagctgtaagttctggggtcttggagcagatggtaccgttggtgctaacaagaactccatcaagatcatcggtgaccacactgacaaatatgctcaggcatactttgattatgattccaagaaatccggtggtgttacaatttcccacttacgtttcggcgatgacccgatcaaagcaacttacctgatcaacaaagctgattttgttgcatgtcactgtgctccgtacatgacaaaatacaacatggttcaggacttaaaagatggcggaacattcttgttaaactgtagctggccggtagaagaaatcggagatcatcttccaggacaggtaaaagcttacatggcaaaacacaacatcaagttctatgtgatcgatggtatcaagatcggtaaagagattggacttggcggacgtatcaatactgtacttcagtctgcattcttcaaattatctggaattattccggaagcagacgcgatccagtatatgaaagacgctgctactgcttcttacagcaagaagggtgatcacatcgttaagatgaatcatgacgcgatcgaagctggtgctaagagtgttgtagaagttccggttcctgctgaatgggctgactgcggagaagaaagcttattacatccagtatccggagatagaaaagatcttgttgattatgttaacaacattcagaacgctgtcaatggacagattggtaacagccttaaggtaagcgacttagttccttacgctgacggtcatatgcctcagggatctgctgcatacgaaaaacgtggagttgctgtagacgttcctacatggaatccggacaactgtatccagtgtaacttctgtgcatatgtatgtcctcatgcagttatccgtcctgttgccatgacagaagcagaacttgctgcagcaccggaagctacaaaatctcttccgatgacgggaatgccagattacaaatttgtaatgacaactactgttcttgactgtacaggatgtggttcttgtgcaaatgtctgcccaggtaagaaaggcgagaaagctcttacaatggcaccactcgacagcatgagagatcagcaggaagtttacaactatggacagtctttacctataaaagaagatatctttgacaagtttaaaccagaatctgttaagggaagccagttcaagaaacctctccttgagttctcaggagcttgtgcaggatgtggagagactccatatgcgaaactgatcactcagttattcggagacagaatgtacattgccaatgcgacaggatgttcttctatctggggtggttcttcacctgcaacaccttacacagtaaacagcgaaggacagggaccggcttggtctaactcactgttcgaagacaatgctgagtttggtttaggtatgttcacaggacagaatactttaagagagcagacaaaagaaaaggttgcagcattagcagaatctacagataatgcagatgtaaaagcagcagcggctgaatacttagatacttacacagacggtaagaaaaacggagcagctactaagaaattagttgcagcactggaagcttgcggatgtgaagaaggaaaagaaatccttaagatgaaagattacttatctaagaaatctcagtggatcttcggtggtgacggatgggcttacgacatcggctttggcggtgttgaccatgtacttgcaagtggtgaagatgttaatatctttgtattcgatacagaggtttactctaacaccggcggacaggcatccaaatctacaccggcaggtgcgatcgctcagttcgcagcagcaggtaaggctgtgaagaaaaaagaccttgcagcaatcgcaatgagctacggatatgtatatgttgctcagatctctatgggtgctgattacaatcagacagtcaaagcgatcgcagaggcagaagcttatccaggaccatcactgatcatcggttatgctccatgtatcaaccacggtatcaagggtggaatgagcattgctcagtctgaagaaaagaaagcagttacatcaggatactggaacttattccgtttcaaccctgaattagctgaagaaggaaagaatccattctcattagattctaaagagcctacaacagagtacaatgacttcatcatgggtgaggttcgttacaacgctcttgctcgccagaatcctgagagagctaaggagctgtttgagcaggcagaaaagaatgccaaagaaaaatatgctcgtttgaaagaattagcagataaataa

SEQ ID NO: 26 - protein, 1174 aa, Anaerostipes rhamnosivorans
MARKMKTMDGNTAAAHVSYAFTETAAIYPITPSSPMAESTDQWATQGKKNIFGHPVKLVEMQSEGGAAGTVHGSLAAGALTTTYTASQGLLLMIPNMYKIAGELMPCVFDVSARAIASHALNIFGDHSDVYACRQTGFAMLCSSSVQEVMDLGAVAHLSTIKGSVPVLHFFDGFRTSHEIQKIEMWDNEDLADMVDYDALEKFRANALNPEHPVLRGSAQNPDIFFQAREACNKYYDAFPAIVEDYMNQVNAKIGTDYKLFNYYGAADAESVIIAMGSVCETIDETIDYLTAKGEKVGVVKVRLYRPFVAEKLLEVIPETVKTINVLDRTKEPGSLGEPLYLDVVSALRGTKFEQVTINGGRYGLGSKDTTPADIISVFNNKDKKEFTVAINDDVTNLSLERGEAVSSTPESTVSCKFWGLGADGTVGANKNSIKIIGDHTDKYAQAYFDYDSKKSGGVTISHLRFGDDPIKATYLINKADFVACHCAPYMTKYNMVQDLKDGGTFLLNCSWPVEEIGDHLPGQVKAYMAKHNIKFYVIDGIKIGKEIGLGGRINTVLQSAFFKLSGIIPEADAIQYMKDAATASYSKKGDHIVKMNHDAIEAGAKSVVEVPVPAEWADCGEESLLHPVSGDRKDLVDYVNNIQNAVNGQIGNSLKVSDLVPYADGHMPQGSAAYEKRGVAVDVPTWNPDNCIQCNFCAYVCPHAVIRPVAMTEAELAAAPEATKSLPMTGMPDYKFVMTTTVLDCTGCGSCANVCPGKKGEKALTMAPLDSMRDQQEVYNYGQSLPIKEDIFDKFKPESVKGSQFKKPLLEFSGACAGCGETPYAKLITQLFGDRMYIANATGCSSIWGGSSPATPYTVNSEGQGPAWSNSLFEDNAEFGLGMFTGQNTLREQTKEKVAALAESTDNADVKAAAAEYLDTYTDGKKNGAATKKLVAALEACGCEEGKEILKMKDYLSKKSQWIFGGDGWAYDIGFGGVDHVLASGEDVNIFVFDTEVYSNTGGQASKSTPAGAIAQFAAAGKAVKKKDLAAIAMSYGYVYVAQISMGADYNQTVKAIAEAEAYPGPSLIIGYAPCINHGIKGGMSIAQSEEKKAVTSGYWNLFRFNPELAEEGKNPFSLDSKEPTTEYNDFIMGEVRYNALARQNPERAKELFEQAEKNAKEKYARLKELADK

SEQ ID NO: 27 - DNA, 1560 bp, Anaerostipes rhamnosivorans
atgggaaaagttaaaattatcacagcagatcaggctgctgccctggtggaggatcatacaacgatcacaaccagcggatttgttgccagcggaatgccggaagctctcacaaaagctttggaaaaaagattcaaagaaaccggatcccccaaaaacctgactttgttttatgctgccgcccagggaaaccgtgacggaagcggcgcggatcattttgcccatgaaggtatgacaaaacgtgtcataggcggacattggaacatggttcctgcactgggacagatggttctggacaataaaatcgaaggctataatctgcctcagggaacactggcacagttataccgtgccatcgcaggtcacaaacccggcgttatcagtcatgtaggattaaatacatttgctgacccacgcattgagggcggtaaattaaatgacattacaaccgaagatatcgtcgatgtagttgaaatcctgggagaagagaaattattgtacaaatcgttcccgatcaacatcggatttatccgcggtacatatgcagatgaacacggcaacgtaactctgtctcacgaatgtgccaccacagaggtcacaaccatggctcaggccgtaaagaacagcggcggaaaggtcgttgtacaggtagaaaaggtcgtttcagacggcaccttagatccaaaattagtcaagatccctggaatttatgtggatgccgttgtggaagtagaagacatgaaggatcacgaacaatgcgtgggctgtgattatgatggttccatgaccggagacttccgggttccgttaagcagtcttgagtacccgcctctttccgccaagaagatcattggacgcagagcagccatggaactgacagaaaacacggttgtaaatctaggcattggtattccagagtacatctccatggtagccaacgaagaaggcattggagattacatgactctgactgtagaggccggaccaatcggcggtgtacctcagggaggagctaaattcggaggcgctgtcaatgctgaatgtatcctagatcagccgtaccagtttgatttctatgacggcggcggagttgactatgcattcttaggactcgcacaggcagataaagacggtaatatcaacgtaagcaagttcggtccaaggattgcgggctgcggcggtttcgtcaatatcacccagaacgcaaaacgctgctacttctgcggaacttttactgcaggaggtctgaagacatccgtaaaagacgggaaacttatcattgaccaggaaggaaaatcaaacaaattcctggataccgtagaacagatcaccttcagcggtgaatacgcaaataaagtcggccagccggttctctatatcacagaacgtgctgtattcgaactcagaaaggacggcgtctatctgacagaggttgcccctggtatcgatatccagacacagatcatcgatcatatgggatttgctccaaagatggaaggaacgccaaagttcatggatgaaagaatcttcaaagatgagctgatgggcctgaagcacgattaa

SEQ ID NO: 28 - protein, 519 aa, Anaerostipes rhamnosivorans
MGKVKIITADQAAALVEDHTTITTSGFVASGMPEALTKALEKRFKETGSPKNLTLFYAAAQGNRDGSGADHFAHEGMTKRVIGGHWNMVPALGQMVLDNKIEGYNLPQGTLAQLYRAIAGHKPGVISHVGLNTFADPRIEGGKLNDITTEDIVDVVEILGEEKLLYKSFPINIGFIRGTYADEHGNVTLSHECATTEVTTMAQAVKNSGGKVVVQVEKVVSDGTLDPKLVKIPGIYVDAVVEVEDMKDHEQCVGCDYDGSMTGDFRVPLSSLEYPPLSAKKIIGRRAAMELTENTVVNLGIGIPEYISMVANEEGIGDYMTLTVEAGPIGGVPQGGAKFGGAVNAECILDQPYQFDFYDGGGVDYAFLGLAQADKDGNINVSKFGPRIAGCGGFVNITQNAKRCYFCGTFTAGGLKTSVKDGKLIIDQEGKSNKFLDTVEQITFSGEYANKVGQPVLYITERAVFELRKDGVYLTEVAPGIDIQTQIIDHMGFAPKMEGTPKFMDERIFKDELMGLKHD

SEQ ID NO: 29 - DNA, 1143 bp, Anaerostipes rhamnosivorans
atgaattttgaattaacagagcagcaggcagccattcaggaaacagcaaggaactttgctcagacagaactgcagccaggtgtgctggagagagatgcaaacagtgagtttccggtagatctttataagaagatgggggatatgggcctgatcggtcttccatatccgaaagaagtcggaggacagggagccgattatctttcttatgcactggcagtggaagagatctcaaaagtagatgcctctgtgggtatttcctattctgtttccacctctctgtatggcggaagcattatgaactctgatgcttccgttgagaaaaagaatgaatttctagcaccggtactgtccggacagcatttcggatcctttggactcacagagcccaatgccggatcagacgcaggcggatgtgtcactgtggctgaaaaagatggggacgaatacatattaaatggtatgaagtgttttaacaccaacggacctttggccgattatacagcggtatatgccctgacagaacctgagaagaaagcaaagggtctttcctgctttgtagtaaaaaaaggaactcctggattttctgtaggcaaggtggaggataagatgggaatccgctctgcgcaggtctctgagatgatcctggaaaatgtcagagtacctgcagagaatatggtcgttccatctggggacggatttaagctggccatgaagactttggatggaggacgcatcggcgttgccgcgcaggggcttggtatcgcggagggcgcatttgagatcgcaaaagaatacttaaagagcagagaacagttcggcaaaccattatataaaaaccagtatcttgcatttaagatggcggaacttgaaatggagatcgacgctgcaagatacatgctttacaaagcggctacagataaacacgagggaagatcttactcaatcccggcagcaaaggcaaaatacctttgtacagaggccgctatgcatgtgacaacagaagcagtacagatgttaggtggaaatgggtatatgaagggttaccatgtagaacgtatgatgagagatgcgaagatcactcagatctatgagggaaccaatgaaatccagaagctcgttgtaagcggagctatcttcagatag

SEQ ID NO: 30 - protein, 380 aa, Anaerostipes rhamnosivorans
MNFELTEQQAAIQETARNFAQTELQPGVLERDANSEFPVDLYKKMGDMGLIGLPYPKEVGGQGADYLSYALAVEEISKVDASVGISYSVSTSLYGGSIMNSDASVEKKNEFLAPVLSGQHFGSFGLTEPNAGSDAGGCVTVAEKDGDEYILNGMKCFNTNGPLADYTAVYALTEPEKKAKGLSCFVVKKGTPGFSVGKVEDKMGIRSAQVSEMILENVRVPAENMVVPSGDGFKLAMKTLDGGRIGVAAQGLGIAEGAFEIAKEYLKSREQFGKPLYKNQYLAFKMAELEMEIDAARYMLYKAATDKHEGRSYSIPAAKAKYLCTEAAMHVTTEAVQMLGGNGYMKGYHVERMMRDAKITQIYEGTNEIQKLVVSGAIFR

SEQ ID NO: 31 - DNA, 777 bp, Anaerostipes rhamnosivorans
atgaacaatttattaatggaagtagaaaacgaagtcgcagttgtaacaatcaacagaccaaaatcattaaacgctttaaacagtgaaactttagctgagttagaccagtgctttacagagatttcaggacgcaaggacatcagagtggtgatcctcacaggatcaggcgaaaaatcctttgtagctggtgctgatatctctgaaatggtcaatgcaactcctgcagaaggaagacagatgggtcttttggcaaaagaagcatttcttaagttagagacaatgcctcaggtaaccatcgctgccgtcaacggttacgctctgggaggcggatgcgagatctccatggcatgtgatatccgtgtagctgcggaaaacgcaaaattcgcacagccagaaacaggacttggaattcttccgggattcggcggaacacagcgtctctcccgtttagtaggaaaaggacgcgcaaaggaattgatctttacatgtgaccagatcgatgccgaagaagcttacagaattggtcttgcaaacaaagtagtgcctcaggcggagctgatcgattactgtaagaagatggctgcaaagatcatgtccaaaggaagctacgcaatttcccttgcaaaagaagcgatcaacacaggaatggacacagacttaagcagcggtcttacattagaagctgacttattcggacttgcattctccactgctgacaaaaaagagggtatgacagcattccttgaaaaacgtaaagctgatttaaaagatttctag

SEQ ID NO: 32 - protein, 258 aa, Anaerostipes rhamnosivorans
MNNLLMEVENEVAVVTINRPKSLNALNSETLAELDQCFTEISGRKDIRVVILTGSGEKSFVAGADISEMVNATPAEGRQMGLLAKEAFLKLETMPQVTIAAVNGYALGGGCEISMACDIRVAAENAKFAQPETGLGILPGFGGTQRLSRLVGKGRAKELIFTCDQIDAEEAYRIGLANKVVPQAELIDYCKKMAAKIMSKGSYAISLAKEAINTGMDTDLSSGLTLEADLFGLAFSTADKKEGMTAFLEKRKADLKDF

SEQ ID NO: 33 - DNA, 1143 bp, Anaerostipes rhamnosivorans
atggttgaatttaaattgacaaaagaacagctgcttgcacagcagatgttcaaagatttcgcagagacagaaatcaagccaattgctagggacatggatgaaacagaagaattcagcatggaactgcttgagaaaatgaaaaaattcggtcttatgggaattccatattccaaagaatacggcggagaaggggcagacgttttaacttatacactctgtatggaagagatgtctaagttagatgcttccacaggaatcacaatttccgtacatacatcattgtgctgttcctgcatcaatgattttgcttcagaagagcagaaacaaaaatttttacgtccgttggttgacggttctaaagtgggatgctttggtcttacagagccgggagcaggtaccgatgccagcggtgtgaagacaaatgccgtattggacggcgatgaatatatcttaaacggacagaaggtgttcactacaaactcaggctttgccgatacatttattatttttgcagttacagacaaaactgcaggtacaagaggtatgtctgcatttatcgtggacaggaatacaccgggattagaagtcagcaagaatatccctcgtatgggtatccgtgctgcgtcaaactgtgaagttgctttagttgatgtgagagtaccgaaggaaaacctgatcgcgggcgagggaaaaggatataagatcgctatgtcagcgctggcaggcggacggatcggaatcggcgctcagtccgtaggaatcgcacagggtgctttaaacgaggccattgcatatgtaaaggaaagaaaacagttcggaaaaccgatttctaaattccagaatacacagttcctgatcgcagaactccaagtgaagatcgacgctgcgcgccttatggtatggagagcggcaaaatcaaaagacgatcatgaaaactatgctcctctggcagcagcgtgcaaactgtttgcatctgacgtggcagtggaagtgacaagagcagccgtacagcttcttggaggatatggatactccagagaatatccggtagagagaatgtaccgtgatgctaagatcacagagatttacgaaggtacatctgaagctatgaagatgatcgtcggcggcggacttttaagataa

SEQ ID NO: 34 - protein, 380 aa, Anaerostipes rhamnosivorans
MVEFKLTKEQLLAQQMFKDFAETEIKPIARDMDETEEFSMELLEKMKKFGLMGIPYSKEYGGEGADVLTYTLCMEEMSKLDASTGITISVHTSLCCSCINDFASEEQKQKFLRPLVDGSKVGCFGLTEPGAGTDASGVKTNAVLDGDEYILNGQKVFTTNSGFADTFIIFAVTDKTAGTRGMSAFIVDRNTPGLEVSKNIPRMGIRAASNCEVALVDVRVPKENLIAGEGKGYKIAMSALAGGRIGIGAQSVGIAQGALNEAIAYVKERKQFGKPISKFQNTQFLIAELQVKIDAARLMVWRAAKSKDDHENYAPLAAACKLFASDVAVEVTRAAVQLLGGYGYSREYPVERMYRDAKITEIYEGTSEAMKMIVGGGLLR

SEQ ID NO: 35 - DNA, 798 bp, Anaerostipes rhamnosivorans
atgaaaatcgttgtttgtgcaaaacaagtaccagatacaactgaagtaaaattagatccaaagaccaacactctgatcagggatggtgttccgagtatcatcaacccagatgacaaagccggaatcgaagctgccctgcagttaaaggaaaaatgcccgggaagcactgtgactgttgtttccatgggaccgcctcaggcagatgtggcattgagagaagcacttgctatgggatgtgacgatgcagttctggtttctgacagagcattcggaggagcagatacatgggcaacatcttccactatcgcggcagcgatcaaaaaattggattacgatgtcatcatcacaggacgccaggcgattgacggagataccgctcaggtaggccctcagatcgcagaacatcttggaattcctcaggtgagctatgtcgaagccctgaatgtggaaggggaagacactttgatcgtccagaggcagtttgaagaccgccatcagatcattgaagtaaagactccttgcctgatcactgctttggctgaattggcaacacctagatatatgacagtccacggtgcatttgacgcatacagagaaaaagaagtcagcgtctggggacttgcagacttagaagacactgtagaccaggcaaatatcgggttaaaaggatctcctacaagagtaaagaaatcctttacaaaacaggccaaaggtgcaggaactattttaaaagatttatcagcagacgaagctgttgcatccattgttgataaacttcaggaaaagcacatcatttaa

SEQ ID NO: 36 - protein, 265 aa, Anaerostipes rhamnosivorans
MKIVVCAKQVPDTTEVKLDPKTNTLIRDGVPSIINPDDKAGIEAALQLKEKCPGSTVTVVSMGPPQADVALREALAMGCDDAVLVSDRAFGGADTWATSSTIAAAIKKLDYDVIITGRQAIDGDTAQVGPQIAEHLGIPQVSYVEALNVEGEDTLIVQRQFEDRHQIIEVKTPCLITALAELATPRYMTVHGAFDAYREKEVSVWGLADLEDTVDQANIGLKGSPTRVKKSFTKQAKGAGTILKDLSADEAVASIVDKLQEKHII

SEQ ID NO: 37 - DNA, 996 bp, Anaerostipes rhamnosivorans
atgagcagagacgtatatgtattcgctgagcagagagacggcgaacttcagaaagtcggaatcgaattaattggtaaagcaagagaattagcagatgatcttggacagcaggtcgttgccgtgctgcttggggcaggcgtaaaagaaaaagcccaggaattagttgcctgcggtgcagataaagttgttgtcgtagatgacattatgctggcagattatgtgacagagccatacacaaaggcactgacagctgtgattaacgcaaaagatcctgagatcgtgctttatggtgcatcttccatcggacgtgaccttgccccaagagtatctgcaaggatccatactggattgacagcggactgtactgcacttgccattgatgaagagacaaagctcctcatgatgacccgtccggcatttggcggaaatatcatggcgaccatcgtgtgtgaagacttccgtcctcagatggcaacagtccgtccaggagtaatgaaagccttggaaaacgatgcatccagaagcggtgaagtggaagagttcaaagtagaattctctgatgcagacatgaatgtaaaagtccgtgaaactgtaaagacagcacataaatctgtagacattacagaggctaagatccttgtttccggtgggcgcggaatcggaagcgctgacaagttcaaggtgttagaggaactggcggatgtcatggaaggtgaagtgtcttcttccagagcatgtgtagattccggatggatcagtgctgaccgccaggtaggacagacaggaaagactgtgcgtccggaattatatctggcctgcggcatctcaggagcgatccagcatgcagccggtatggagaactcagagtttatcgtagccatcaaccgtgatgaggatgcgccgatctttgatattgcagacctcggcatcgttggagacttaaataccatcgtaccgaaacttacagaagctgtgaaggcggtaaaaggaaaataa

SEQ ID NO: 38 - protein, 331 aa, Anaerostipes rhamnosivorans
MSRDVYVFAEQRDGELQKVGIELIGKARELADDLGQQVVAVLLGAGVKEKAQELVACGADKVVVVDDIMLADYVTEPYTKALTAVINAKDPEIVLYGASSIGRDLAPRVSARIHTGLTADCTALAIDEETKLLMMTRPAFGGNIMATIVCEDFRPQMATVRPGVMKALENDASRSGEVEEFKVEFSDADMNVKVRETVKTAHKSVDITEAKILVSGGRGIGSADKFKVLEELADVMEGEVSSSRACVDSGWISADRQVGQTGKTVRPELYLACGISGAIQHAAGMENSEFIVAINRDEDAPIFDIADLGIVGDLNTIVPKLTEAVKAVKGK

SEQ ID NO: 39 - DNA, 834 bp, Anaerostipes rhamnosivorans
atgaaaatcggatttaacgaagcaactgcactggaatgtaaaggacagtctctgatggctgacttagaagcgtgtgaaaaatacggatttgattacatcgagatcagatttgactgtgtaaaggattatttgaaagaacacacactggaagaactggcggactggtttaaaaaccatcatttaaaaccatgggcttataataccttgatcttttttaaccagagagacgaagccggagaaaaagagattgacgaagagactgattttatcattgaagtgtgcaaggccatcggcatgaagatgctgatcactgttccgtcctttgatgtaaaggataagagcatcacagagatcaaagaggaagcagtagaacgtctccgttatttatccgataaggtgggagaagatattaagatatcactggaattctgcggggcgccgaactgctccatcaaccagtttgggacagcttacgatgtagtgaaagcaacagaccgtgacaatgtaggggtaacagtggataccttccatttccatgagatgtgttctaagttagaagatttagaagcagcggacggaaagaagatctttgcttaccatctgaatgactgtgaggatctgcctctgggatcatgcggtgatgataaacgcctgtggccgggagaaggtgtggtagatcatgcaggaatcgcagctgccttaaagaagatcggattcgacggggtatgtaccattgaagaattccgtccagaatattatgaaatgtcccatgacgagaatgtgaaaaagtctgctgaagtgacaagggatttcgtagcaaaatactttgcataa

SEQ ID NO: 40 - protein, 277 aa, Anaerostipes rhamnosivorans
MKIGFNEATALECKGQSLMADLEACEKYGFDYIEIRFDCVKDYLKEHTLEELADWFKNHHLKPWAYNTLIFFNQRDEAGEKEIDEETDFIIEVCKAIGMKMLITVPSFDVKDKSITEIKEEAVERLRYLSDKVGEDIKISLEFCGAPNCSINQFGTAYDVVKATDRDNVGVTVDTFHFHEMCSKLEDLEAADGKKIFAYHLNDCEDLPLGSCGDDKRLWPGEGVVDHAGIAAALKKIGFDGVCTIEEFRPEYYEMSHDENVKKSAEVTRDFVAKYFA

SEQ ID NO: 41 - DNA, 945 bp, Anaerostipes rhamnosivorans
atgacatataaaatgagaaaaatagtgatcataggggccggacatgtgggaaccatgtgcggcctgagtcttatgtaccgcggagaagtggacgaattggtattcatagacatcgataaggaaaaggcatacagccaggcgctggaccttagtgatgccgtctccttcctgccccggcagatcacggtgcgcaccggggattatgaagatgtggaggacgctgacatcatcgttatggccgctggtgtttccaggctgcccggtcagacaaggctggatatgctggacgattccatccgcatcatgaaagaagtcaccagccatttaaaagataagaagattcagggcatcctcatcagtatctccaatcctgccgacattgtggcggattatctgagaaaacaactgggccttccgagaaaccgctgcttcagcaccggtacttccctggactcctgccgtctcagaaggattctttcccaaagaatgcacttagaccggaattccattcaggcctttgtcatgggagaacacggagattcccaaatgatcccgttttctgcggtacatatagccgggaaaccattgcttcagtggatgcaagatgaaccggaacggtacggaagtctcgatctttcacagattgaaacggagaccgccaacgccggccatgaagtgatcgaaggaaagggcagcacagagtttggtatcggcatcgccctgtccgagatcgtccagtccattttccacgattcaaaaaaggtccttcccgcttcgcctctgctggaaggagaatatggacagcatggcgttcacgccggtgtcccctgcgtgattggaaaagccggaattgaaaagatcattgagatccctctcacagaccgggagcaagagaaatttgaccattcctgcgatgtgatcagaacgtttattcaagatctctga

SEQ ID NO: 42 - protein, 314 aa, Anaerostipes rhamnosivorans
MTYKMRKIVIIGAGHVGTMCGLSLMYRGEVDELVFIDIDKEKAYSQALDLSDAVSFLPRQITVRTGDYEDVEDADIIVMAAGVSRLPGQTRLDMLDDSIRIMKEVTSHLKDKKIQGILISISNPADIVADYLRKQLGLPRNRCFSTGTSLDSCRLRRILSQRMHLDRNSIQAFVMGEHGDSQMIPFSAVHIAGKPLLQWMQDEPERYGSLDLSQIETETANAGHEVIEGKGSTEFGIGIALSEIVQSIFHDSKKVLPASPLLEGEYGQHGVHAGVPCVIGKAGIEKIIEIPLTDREQEKFDHSCDVIRTFIQDL

SEQ ID NO: 43 - DNA, 1176 bp, Anaerostipes rhamnosivorans
atgggaagatttacattacctagagatttgtactttggaaaaggatcacttgagacactgaagacgctggacggaaaaaaagctgttttagtcatcggcggcggatctatgaaacgttttggatttgtagaccaggttgttgattatttaaaagaagcaggcatagagacaaaattaattgagggagtagagccggacccttctgttgagaccgtatttaaaggtgccgagattatgagagagtttgaaccggactggatcgtggcaatgggcggaggatctccgatcgatgctgcaaaagctatgtggatcttctatgaacatccggaaaccacatttgacgatgtaaaagacccattcacagttccaaaactcagaaacaaagcaagattccttgcaatcccttcaacttcaggaacagctacggaagtgacggcatttgctgttatcacggactacagttcaggcattaaatatccgctggcagactttgagatcacaccggatgttgccattgtagaccctgcactggcagagacgatgcctccgaaactgacctcttatacaggaatggatgcactgacccatgcgattgaagcatatgttgccggactgcattcaccattttcagatcctttggcaatcgatgccatcgagatggtatttgacaacttaaaagcttcctatgagggagacatgaccgcacgtgaaaatatgcactatgcacaatgtcttgcaggaatgtcattctctaatgcactgttaggaattgtacattctttagcgcataagacaggagcagtttttgatacaggacatatcacacacggatgtgcgaacgctatctatcttccgtatgtgatccagtttaatgcaaaggtatgcgaagaccgctatgcagccattgcaagaaagatcggcctccctggaaattccgataaagcactgacactttctttgattgaagcaatccgggatatgaacaagaagctgaacattgtttccaacctgaaagatttcggaatcaatgaagaagaattcaaccagaagaagaggatgatcgcggagcgtgctgtggcagacgcatgtacaggatctaatcctagagaaacctctgtagatgacatggaaaaagtgttagagtgcatctactacggaaaagacgtaatattctaa

SEQ ID NO: 44 - protein, 391 aa, Anaerostipes rhamnosivorans
MGRFTLPRDLYFGKGSLETLKTLDGKKAVLVIGGGSMKRFGFVDQVVDYLKEAGIETKLIEGVEPDPSVETVFKGAEIMREFEPDWIVAMGGGSPIDAAKAMWIFYEHPETTFDDVKDPFTVPKLRNKARFLAIPSTSGTATEVTAFAVITDYSSGIKYPLADFEITPDVAIVDPALAETMPPKLTSYTGMDALTHAIEAYVAGLHSPFSDPLAIDAIEMVFDNLKASYEGDMTARENMHYAQCLAGMSFSNALLGIVHSLAHKTGAVFDTGHITHGCANAIYLPYVIQFNAKVCEDRYAAIARKIGLPGNSDKALTLSLIEAIRDMNKKLNIVSNLKDFGINEEEFNQKKRMIAERAVADACTGSNPRETSVDDMEKVLECIYYGKDVIF

SEQ ID NO: 45 - DNA, 1184 bp, Anaerostipes rhamnosivorans
cgaaagtccgtgaatttttgtgccttaccgcacatcctcagggctgcagaaaaaatgttgaagatcagattacatatgtaaaaaaacacagcggtgttgagaatgggccgaaaaaggtcctggtcatcggctcatccacgggatatggcctggcatcaaggatcaccgctgcattcgggtgcggagcggataccttgggtgtcatgtttgagagaccggcggccggtaaacgtaccgccactgccggatggtataatacagctgcatttgaacaggcggcggccagagaaggcttatatgcgaagacggtcaacgcagatgcattttccagggaagtaaaagaccaggtcatccaactgatcaagaaggatttcggtaaggttgacgctgtcatttacagtctggctgcaccgagaagaacgacagaggacggcacggtttatcagtctgtcttaaagacaacaggggaagattttacaaataagaacctgaaccttaaagataataccatcagtgagaaaaccatcgaggctgccacagaggaagaagtgaaagctaccgtgaaggtcatgggcggggaggactggaaggcatggatccaggcgcttaccgatgcggatgccattgaaaagggcgcagtcaccttcgcatattcttatatcggacctaagcttacatatcctatctattttgagggaaccatcggtgccgcgaagaagcatcttcataagacggcgggtgagatcaatgaggaattctcaaaggatggaatcaaagcatacatctccgtcaataaggggctggtgacacaggccagttctgccattccgatcgtaccgctttatatggctgtgctgtaccgcgttatgaaagaaaagggacttcatgaaggctgtatcgaacagatcgtaaggctgttttctgaaaaggctgtctttggacaggccaagacagatgaacagggtctgatccgtctggatgactgggaactgcgcccggaagtccaggaagaagtggaacgccgctgggagaaggtctgcaccgaaaatgtccaggagtattctgatattgacggatactgggatgatttctaccaaatgttcggcttccgtatggatggagtggactacgaggaggatcttgacccttctgtggatatcccaagcatttccggccaagaatag

SEQ ID NO: 46 - protein, 398 aa, Anaerostipes rhamnosivorans
MKISPKVREFLCLTAHPQGCRKNVEDQITYVKKHSGVENGPKKVLVIGSSTGYGLASRITAAFGCGADTLGVMFERPAAGKRTATAGWYNTAAFEQAAAREGLYAKTVNADAFSREVKDQVIQLIKKDFGKVDAVIYSLAAPRRTTEDGTVYQSVLKTTGEDFTNKNLNLKDNTISEKTIEAATEEEVKATVKVMGGEDWKAWIQALTDADAIEKGAVTFAYSYIGPKLTYPIYFEGTIGAAKKHLHKTAGEINEEFSKDGIKAYISVNKGLVTQASSAIPIVPLYMAVLYRVMKEKGLHEGCIEQIVRLFSEKAVFGQAKTDEQGLIRLDDWELRPEVQEEVERRWEKVCTENVQEYSDIDGYWDDFYQMFGFRMDGVDYEEDLDPSVDIPSISGQE

SEQ ID NO: 47 - DNA, 1434 bp, Anaerostipes rhamnosivorans
atgctgacaaaaaaaacaaagattgtttgcacgatggggcctgcgacagatgatgatgcggtgctcaaacagctgatgctggaaggaatggatatcgcgaggctgaatttctctcacggtgaccatgaggaacagcttggaaggatcaagagaattaaaagattccgtgaagaactgaatattccgatcgcgatcttactggatacaaaaggacctgagatccgtacaggacttctggagacagacggagacgtggaattaaaagaaggaaatgaatttgttctgaccacaagggacatcaaaggaaatgattctatcgtagcaattacatacgaagagcttccgcaggatgtcacagaaggaaatacaatcctgatcgatgacggtctgatcgaactgagagtcaaagagatcaaagacggaacagatattgtatgtgaaattgtaaacggcggacttttaggaagccgtaagggagtgaacgtaccgaacgtgcgcgtaaatcttccttccatcacagaaaaggataagagagacattgagttcggacttgaaaacggcattgattttatcgcggcttctttcatccgtaacgcagatgcagtcaatgagatcaaggacatcgtaaaagcccacaacatggaagtcggcgttatctccaaaattgaaaacgtggagggtgtggaaaatattgaatccatcatccaggcttctgacggaatcatggtagcccgtggagatttaggtgtggaaattcccgcagaggaagttccgtttatgcagaaagcaatcattaagaaatgcaacaatgcatttaagccagtcatcacagctacacagatgttagactctatgatcagaaacccacgtccgacaagagcggaagtaacagacgttgccaatgctatttatgacggaaccgatgcgattatgctttctggagaaaccgcgaaggggaaataccctgtggaggccgtaaggatgatgaaccagatcgccatctccacagaactgcatctggatacgaagatcaaagattttcgttccatctatgtaagccgtggaatctcagcagcggttgcttattctgctgtacagactgctcataatattaacgcaaaatgtatcctggcgtccagtatgtccggatttacggcaaggatcgtatctaagttcaaaccggatgcacagatcattggcttgtctccggatgaagcggttgtgcgtaagatgcagctttactggggagtgcgtccgtttaagtcacataaggcttcctctaccagagaacttttggatgaagctacggatatcgtactgaatgcagatcttgcacaggagaacgacatcctggtactgaccggaggaggtccggcagaccaccgtggaaaaggcgtgacaaacatgctgaaagtagtaaaaatcggcgaataa

SEQ ID NO: 48 - protein, 477 aa, Anaerostipes rhamnosivorans
MLTKKTKIVCTMGPATDDDAVLKQLMLEGMDIARLNFSHGDHEEQLGRIKRIKRFREELNIPIAILLDTKGPEIRTGLLETDGDVELKEGNEFVLTTRDIKGNDSIVAITYEELPQDVTEGNTILIDDGLIELRVKEIKDGTDIVCEIVNGGLLGSRKGVNVPNVRVNLPSITEKDKRDIEFGLENGIDFIAASFIRNADAVNEIKDIVKAHNMEVGVISKIENVEGVENIESIIQASDGIMVARGDLGVEIPAEEVPFMQKAIIKKCNNAFKPVITATQMLDSMIRNPRPTRAEVTDVANAIYDGTDAIMLSGETAKGKYPVEAVRMMNQIAISTELHLDTKIKDFRSIYVSRGISAAVAYSAVQTAHNINAKCILASSMSGFTARIVSKFKPDAQIIGLSPDEAVVRKMQLYWGVRPFKSHKASSTRELLDEATDIVLNADLAQENDILVLTGGGPADHRGKGVTNMLKVVKIGE